European Patent Application EP 4 603 498 A1, published August 20, 2025. Title: Peptide Having Activity of Promoting Hair Growth and Inhibiting Hair Loss and Uses Thereof. Applicant: CAREGENE CO., LTD. Application KR. The sequence listing filed with the application follows.

SEQUENCE LISTING (9 sequences)

SEQ ID NO: 1 - protein, 4 aa, synthetic construct
LAMD

SEQ ID NO: 2 - DNA, 20 bp, synthetic construct
  source 1..20: mol_type = other DNA
tgctggtgatgggagttgta

SEQ ID NO: 3 - DNA, 20 bp, synthetic construct
  source 1..20: mol_type = other DNA
cctccaagtagcagccaaag

SEQ ID NO: 4 - DNA, 22 bp, synthetic construct
  source 1..22: mol_type = other DNA
tctgtcgaacacagtggtacct

SEQ ID NO: 5 - DNA, 23 bp, synthetic construct
  source 1..23: mol_type = other DNA
gtgtgtccatttagctgatgcat

SEQ ID NO: 6 - DNA, 23 bp, synthetic construct
  source 1..23: mol_type = other DNA
atgaactttctgctgtcttgggt

SEQ ID NO: 7 - DNA, 22 bp, synthetic construct
  source 1..22: mol_type = other DNA
tggccttggtgaggtttgatcc

SEQ ID NO: 8 - DNA, 20 bp, synthetic construct
  source 1..20: mol_type = other DNA
ggagccaaaagggtcatcat

SEQ ID NO: 9 - DNA, 20 bp, synthetic construct
  source 1..20: mol_type = other DNA
gtgatggcatggactgtggt